European Patent Application EP 4 497 755 A1, published January 29, 2025. Title: THERAPEUTIC ANTIBODIES. Applicant: ASOCIACIÓN CENTRO DE INVESTIGACIÓN COOPERATIVA EN BIOCENCIAS-CIC bioGUNE. Application EP. The sequence listing filed with the application follows.

SEQUENCE LISTING (146 sequences)

SEQ ID NO: 1 - protein, 6 aa, synthetic construct
LLDLER

SEQ ID NO: 2 - protein, 8 aa, synthetic construct
LLDLERGT

SEQ ID NO: 3 - protein, 12 aa, synthetic construct
LLDLERGTRESA

SEQ ID NO: 4 - protein, 10 aa, synthetic construct
GFTFSDYGMA

SEQ ID NO: 5 - protein, 17 aa, synthetic construct
SITSGGGNPYYRDSVKG

SEQ ID NO: 6 - protein, 13 aa, synthetic construct
HEYYGNYMTCFDY

SEQ ID NO: 7 - protein, 12 aa, synthetic construct
RASLSISSNYLH

SEQ ID NO: 8 - protein, 7 aa, synthetic construct
STSYRAS

SEQ ID NO: 9 - protein, 9 aa, synthetic construct
QQGSSDPLT

SEQ ID NO: 10 - protein, 10 aa, synthetic construct
GFTFSNYGMA

SEQ ID NO: 11 - protein, 17 aa, synthetic construct
SINYDGRNTYYRDSVKG

SEQ ID NO: 12 - protein, 8 aa, synthetic construct
PQDGVIDA

SEQ ID NO: 13 - protein, 16 aa, synthetic construct
RSSQSLVHSNGNTYLH

SEQ ID NO: 14 - protein, 7 aa, synthetic construct
RVSNRFS

SEQ ID NO: 15 - protein, 9 aa, synthetic construct
LQGTHLPPT

SEQ ID NO: 16 - protein, 122 aa, synthetic construct
EVELVESGGGLVQPGRSLKLSCAASGFTFSDYGMAWVRQTPTKGLEWVASITSGGGNPYYRDSVKGRFTISRDNAKNTQHLQMDSLRSEDTATYYCARHEYYGNYMTCFDYWGQGVMVTVSS

SEQ ID NO: 17 - protein, 108 aa, synthetic construct
AIVLNQSPSSIVASQGEKVTITCRASLSISSNYLHWYQQKPGAFPKLVIYSTSYRASGVPSRFSGSGSGTSYSFTISRVEAEDVATYYCQQGSSDPLTFGSGTKLEIK

SEQ ID NO: 18 - protein, 117 aa, synthetic construct
EVQLVESGGGLVQPGRSLKLSCAASGFTFSNYGMAWVRQAPTKGLEWVASINYDGRNTYYRDSVKGRFTISRDNAKSTVYLQMDSLRSEDTATYYCARPQDGVIDAWGQGDSVTVSS

SEQ ID NO: 19 - protein, 112 aa, synthetic construct
DVVMTQTPVSLPVSLGGQASISCRSSQSLVHSNGNTYLHWYLQKPGQFPQLLIYRVSNRFSGVPDRFSGSGSGTDFTLKISRVESEDLGVYYCLQGTHLPPTFGGGTKLELK

SEQ ID NO: 20 - protein, 327 aa, synthetic construct
ASTKGPSVFPLAPCSRSTSESTAALGCLVKDYFPEPVTVSWNSGALTSGVHTFPAVLQSSGLYSLSSVVTVPSSSLGTKTYTCNVDHKPSNTKVDKRVESKYGPPCPPCPAPEFLGGPSVFLFPPKPKDTLMISRTPEVTCVVVDVSQEDPEVQFNWYVDGVEVHNAKTKPREEQFNSTYRVVSVLTVLHQDWLNGKEYKCKVSNKGLPSSIEKTISKAKGQPREPQVYTLPPSQEEMTKNQVSLTCLVKGFYPSDIAVEWESNGQPENNYKTTPPVLDSDGSFFLYSRLTVDKSRWQEGNVFSCSVMHEALHNHYTQKSLSLSLGK

SEQ ID NO: 21 - protein, 107 aa, synthetic construct [sequence omitted]

SEQ ID NO: 22 - protein, 449 aa, synthetic construct
EVELVESGGGLVQPGRSLKLSCAASGFTFSDYGMAWVRQTPTKGLEWVASITSGGGNPYYRDSVKGRFTISRDNAKNTQHLQMDSLRSEDTATYYCARHEYYGNYMTCFDYWGQGVMVTVSSASTKGPSVFPLAPCSRSTSESTAALGCLVKDYFPEPVTVSWNSGALTSGVHTFPAVLQSSGLYSLSSVVTVPSSSLGTKTYTCNVDHKPSNTKVDKRVESKYGPPCPPCPAPEFLGGPSVFLFPPKPKDTLMISRTPEVTCVVVDVSQEDPEVQFNWYVDGVEVHNAKTKPREEQFNSTYRVVSVLTVLHQDWLNGKEYKCKVSNKGLPSSIEKTISKAKGQPREPQVYTLPPSQEEMTKNQVSLTCLVKGFYPSDIAVEWESNGQPENNYKTTPPVLDSDGSFFLYSRLTVDKSRWQEGNVFSCSVMHEALHNHYTQKSLSLSLGK

SEQ ID NO: 23 - protein, 215 aa, synthetic construct
AIVLNQSPSSIVASQGEKVTITCRASLSISSNYLHWYQQKPGAFPKLVIYSTSYRASGVPSRFSGSGSGTSYSFTISRVEAEDVATYYCQQGSSDPLTFGSGTKLEIKRTVAAPSVFIFPPSDEQLKSGTASVVCLLNNFYPREAKVQWKVDNALQSGNSQESVTEQDSKDSTYSLSSTLTLSKADYEKHKVYACEVTHQGLSSPVTKSFNRGEC

SEQ ID NO: 24 - protein, 12 aa, synthetic construct
LLAAERGTRESA

SEQ ID NO: 25 - protein, 8 aa, synthetic construct
GPVLDKAT

SEQ ID NO: 26 - protein, 122 aa, synthetic construct
QVQLVESGGGVVQPGRSLRLSCAASGFTFSDYGMAWVRQAPGKGLEWVASITSGGGNPYYRDSVKGRFTISRDNSKNTLYLQMNSLRAEDTAVYYCARHEYYGNYMTCFDYWGQGTLVTVSS

SEQ ID NO: 27 - protein, 122 aa, synthetic construct
QVQLVESGGGVVQPGRSLRLSCAASGFTFSDYGMAWVRQAPGKGLEWVASITSGGGNPYYRDSVKGRFTISRDNAKNTLYLQMNSLRAEDTAVYYCARHEYYGNYMTCFDYWGQGTLVTVSS

SEQ ID NO: 28 - protein, 141 aa, synthetic construct
MDFRLSLAFLVLLIKGVQCEVELVESGGGLVQPGRSLKLSCAASGFTFSDYGMAWVRQTPTKGLEWVASITSGGGNPYYRDSVKGRFTISRDNAKNTQHLQMDSLRSEDTATYYCARHEYYGNYMTCFDYWGQGVMVTVSS

SEQ ID NO: 29 - protein, 128 aa, synthetic construct
MNFQVQVFSFLLISVSVSSGAIVLNQSPSSIVASQGEKVTITCRASLSISSNYLHWYQQKPGAFPKLVIYSTSYRASGVPSRFSGSGSGTSYSFTISRVEAEDVATYYCQQGSSDPLTFGSGTKLEIK

SEQ ID NO: 30 - protein, 136 aa, synthetic construct
MDIRLSLVFLVLFIKGVQCEVQLVESGGGLVQPGRSLKLSCAASGFTFSNYGMAWVRQAPTKGLEWVASINYDGRNTYYRDSVKGRFTISRDNAKSTVYLQMDSLRSEDTATYYCARPQDGVIDAWGQGDSVTVSS

SEQ ID NO: 31 - protein, 131 aa, synthetic construct
MKWPVRLLVLFFWIPASRGDVVMTQTPVSLPVSLGGQASISCRSSQSLVHSNGNTYLHWYLQKPGQFPQLLIYRVSNRFSGVPDRFSGSGSGTDFTLKISRVESEDLGVYYCLQGTHLPPTFGGGTKLELK

SEQ ID NO: 32 - protein, 330 aa, synthetic construct [sequence omitted]

SEQ ID NO: 33 - protein, 122 aa, synthetic construct
QVQLVESGGGVVQPGRSLRLSCAASGFTFSDYGMAWVRQAPGKGLEWVASITSGGGNPYYRDSVKGRFTISRDNSKNTQHLQMNSLRAEDTAVYYCARHEYYGNYMTCFDYWGQGTLVTVSS

SEQ ID NO: 34 - protein, 122 aa, synthetic construct
QVQLVESGGGVVQPGRSLRLSCAASGFTFSDYGMAWVRQAPGKGLEWVASITSGGGNPYYRDSVKGRFTISRDNAKNTQHLQMNSLRAEDTAVYYCARHEYYGNYMTCFDYWGQGTLVTVSS

SEQ ID NO: 35 - protein, 12 aa, synthetic construct
LLALERGTRESA

SEQ ID NO: 36 - protein, 12 aa, synthetic construct
LLDAERGTRESA

SEQ ID NO: 37 - protein, 20 aa, synthetic construct
GGTTCTCTCCATCGCCTTGT

SEQ ID NO: 38 - protein, 21 aa, synthetic construct
GGAATGCTTCTCACACTCCCA

SEQ ID NO: 39 - protein, 4 aa, synthetic construct
APNY

SEQ ID NO: 40 - protein, 8 aa, synthetic construct
LLDLERGT

SEQ ID NO: 41 - protein, 4 aa, synthetic construct
RESA

SEQ ID NO: 42 - DNA, 18 bp, synthetic construct
  source 1..18: mol_type = other DNA
cgggagtcggccttcgtg

SEQ ID NO: 43 - DNA, 18 bp, synthetic construct
  source 1..18: mol_type = other DNA
atagttgggggcgagctc

SEQ ID NO: 44-46 - skipped (3 entries)

SEQ ID NO: 47 - protein, 12 aa, synthetic construct
GVAMPGAEDDVV

SEQ ID NO: 48 - protein, 14 aa, synthetic construct
GKPIPNPLLGLDST

SEQ ID NO: 49 - protein, 11 aa, synthetic construct
YTDIEMNRLGK

SEQ ID NO: 50 - DNA, 20 bp, synthetic construct
  source 1..20: mol_type = other DNA
gtgttcgacaatggcagcat

SEQ ID NO: 51 - DNA, 21 bp, synthetic construct
  source 1..21: mol_type = other DNA
agacactggcaacattgcgga

SEQ ID NO: 52 - DNA, 20 bp, synthetic construct
  source 1..20: mol_type = other DNA
tgagggtctgcgtgaaatcc

SEQ ID NO: 53 - DNA, 20 bp, synthetic construct
  source 1..20: mol_type = other DNA
tgggaacaacccccattgtc

SEQ ID NO: 54 - DNA, 20 bp, synthetic construct
  source 1..20: mol_type = other DNA
gctctacaaccgcgtcaaga

SEQ ID NO: 55 - DNA, 20 bp, synthetic construct
  source 1..20: mol_type = other DNA
gctgaaaaaggggttgtggc

SEQ ID NO: 56 - DNA, 20 bp, synthetic construct
  source 1..20: mol_type = other DNA
tgaaggactcggaactcgtc

SEQ ID NO: 57 - DNA, 20 bp, synthetic construct
  source 1..20: mol_type = other DNA
gtcgcttccgttggatgtct

SEQ ID NO: 58 - DNA, 18 bp, synthetic construct
  source 1..18: mol_type = other DNA
ctcctcctgggtgtgacc

SEQ ID NO: 59 - DNA, 20 bp, synthetic construct
  source 1..20: mol_type = other DNA
cagtgttgcgtctggttcag

SEQ ID NO: 60 - DNA, 20 bp, synthetic construct
  source 1..20: mol_type = other DNA
aagtgcaaactttcgccaac

SEQ ID NO: 61 - DNA, 20 bp, synthetic construct
  source 1..20: mol_type = other DNA
acaggatcgctcctcttgaa

SEQ ID NO: 62 - DNA, 19 bp, synthetic construct
  source 1..19: mol_type = other DNA
acttccagccgaaagtcgt

SEQ ID NO: 63 - DNA, 18 bp, synthetic construct
  source 1..18: mol_type = other DNA
caccataggccgaagcac

SEQ ID NO: 64 - DNA, 20 bp, synthetic construct
  source 1..20: mol_type = other DNA
agcacggaaagaaagacagc

SEQ ID NO: 65 - DNA, 21 bp, synthetic construct
  source 1..21: mol_type = other DNA
tcgttttccacctgatgcaga

SEQ ID NO: 66 - DNA, 19 bp, synthetic construct
  source 1..19: mol_type = other DNA
atgcgtcacgctatgtgct

SEQ ID NO: 67 - DNA, 20 bp, synthetic construct
  source 1..20: mol_type = other DNA
tctggaatacccatccaagg

SEQ ID NO: 68 - DNA, 20 bp, synthetic construct
  source 1..20: mol_type = other DNA
gatgtgggctgtgcagtttg

SEQ ID NO: 69 - DNA, 22 bp, synthetic construct
  source 1..22: mol_type = other DNA
agtcctttacctcacccagagt

SEQ ID NO: 70 - DNA, 17 bp, synthetic construct
  source 1..17: mol_type = other DNA
gtcaccagaacttgtgc

SEQ ID NO: 71 - DNA, 18 bp, synthetic construct
  source 1..18: mol_type = other DNA
caaagatgctgttcatgg

SEQ ID NO: 72 - DNA, 23 bp, synthetic construct
  source 1..23: mol_type = other DNA
gcccactttctcctaccaatacc

SEQ ID NO: 73 - DNA, 17 bp, synthetic construct
  source 1..17: mol_type = other DNA
ctccggctgccctcact

SEQ ID NO: 74 - DNA, 25 bp, synthetic construct
  source 1..25: mol_type = other DNA
tgctgcgagtaggacatgctgtagg

SEQ ID NO: 75 - DNA, 23 bp, synthetic construct
  source 1..23: mol_type = other DNA
gcacatgaacggctggagcaacg

SEQ ID NO: 76 - protein, 13 aa, synthetic construct
LLDLERGTRESAC

SEQ ID NO: 77 - protein, 12 aa, synthetic construct
ALDLERGTRESA

SEQ ID NO: 78 - protein, 12 aa, synthetic construct
LADLERGTRESA

SEQ ID NO: 79 - protein, 12 aa, synthetic construct
LLDLARGTRESA

SEQ ID NO: 80 - protein, 12 aa, synthetic construct
LLDLEAGTRESA

SEQ ID NO: 81 - protein, 12 aa, synthetic construct
LLDLERATRESA

SEQ ID NO: 82 - protein, 12 aa, synthetic construct
LLDLERGARESA

SEQ ID NO: 83 - protein, 12 aa, synthetic construct
LLDLERGTAESA

SEQ ID NO: 84 - protein, 12 aa, synthetic construct
LLDLERGTRASA

SEQ ID NO: 85 - protein, 12 aa, synthetic construct
LLDLERGTREAA

SEQ ID NO: 86 - protein, 12 aa, synthetic construct
AADLERGTRESA

SEQ ID NO: 87 - protein, 12 aa, synthetic construct
LLAAERGTRESA

SEQ ID NO: 88 - protein, 12 aa, synthetic construct
LLDLAAGTRESA

SEQ ID NO: 89 - protein, 12 aa, synthetic construct
LLDLERAARESA

SEQ ID NO: 90 - protein, 12 aa, synthetic construct
LLDLERGTAASA

SEQ ID NO: 91 - protein, 12 aa, synthetic construct
AAAAERGTRESA

SEQ ID NO: 92 - protein, 12 aa, synthetic construct
LLDLAAAARESA

SEQ ID NO: 93 - protein, 12 aa, synthetic construct
LLDLERGTAAAA

SEQ ID NO: 94 - protein, 12 aa, synthetic construct
GPVLDKATRESA

SEQ ID NO: 95 - protein, 7 aa, synthetic construct
LLDLERG

SEQ ID NO: 96 - DNA, 24 bp, synthetic construct
  source 1..24: mol_type = other DNA
gacctcgagagagggacccgggag

SEQ ID NO: 97 - DNA, 24 bp, synthetic construct
  source 1..24: mol_type = other DNA
aagcgcatagttgggggcgagctc

SEQ ID NO: 98 - DNA, 22 bp, synthetic construct
  source 1..22: mol_type = other DNA
cctcgagagagggacccgggag

SEQ ID NO: 99 - DNA, 24 bp, synthetic construct
  source 1..24: mol_type = other DNA
tcagccaaatagttgggggcgagc

SEQ ID NO: 100 - DNA, 28 bp, synthetic construct
  source 1..28: mol_type = other DNA
ctatttgcttgccctcgagagagggacc

SEQ ID NO: 101 - DNA, 18 bp, synthetic construct
  source 1..18: mol_type = other DNA
ttgggggcgagctcaatg

SEQ ID NO: 102 - DNA, 24 bp, synthetic construct
  source 1..24: mol_type = other DNA
agaggtacccgggagtcggccttc

SEQ ID NO: 103 - DNA, 28 bp, synthetic construct
  source 1..28: mol_type = other DNA
ctccgcgtcaagcaaatagttgggggcg

SEQ ID NO: 104 - DNA, 22 bp, synthetic construct
  source 1..22: mol_type = other DNA
aggtacccgggagtcggccttc

SEQ ID NO: 105 - DNA, 28 bp, synthetic construct
  source 1..28: mol_type = other DNA
ctcgccaggtcaagcaaatagttggggg

SEQ ID NO: 106 - DNA, 24 bp, synthetic construct
  source 1..24: mol_type = other DNA
gaagggacccgggagtcggccttc

SEQ ID NO: 107 - DNA, 28 bp, synthetic construct
  source 1..28: mol_type = other DNA
ctcgaggtcaagcaaatagttgggggcg

SEQ ID NO: 108 - DNA, 25 bp, synthetic construct
  source 1..25: mol_type = other DNA
agcgacccgggagtcggccttcgtg

SEQ ID NO: 109 - DNA, 29 bp, synthetic construct
  source 1..29: mol_type = other DNA
ctctcgaggtcaagcaaatagttgggggc

SEQ ID NO: 110 - protein, 108 aa, synthetic construct
DIQMTQSPSSLSASVGDRVTITCRASLSISSNYLHWYQQKPGKAPKLLIYSTSYRASGVPSRFSGSGSGTDFTLTISSLQPEDFATYYCQQGSSDPLTFGGGTKLEIK

SEQ ID NO: 111 - protein, 108 aa, synthetic construct
DIQMTQSPSSLSASVGDRVTITCRASLSISSNYLHWYQQKPGKAPKLVIYSTSYRASGVPSRFSGSGSGTDFTLTISSLQPEDFATYYCQQGSSDPLTFGGGTKLEIK

SEQ ID NO: 112 - protein, 108 aa, synthetic construct
DIQMTQSPSSLSASVGDRVTITCRASLSISSNYLHWYQQKPGKAPKLVIYSTSYRASGVPSRFSGSGSGTDYTLTISSLQPEDFATYYCQQGSSDPLTFGGGTKLEIK

SEQ ID NO: 113 - protein, 108 aa, synthetic construct
DIQMTQSPSSLSASQGDRVTITCRASLSISSNYLHWYQQKPGKAPKLVIYSTSYRASGVPSRFSGSGSGTDYTLTISSLQPEDFATYYCQQGSSDPLTFGGGTKLEIK

SEQ ID NO: 114 - protein, 366 aa, Homo sapiens
MRARPQVCEALLFALALQTGVCYGIKWLALSKTPSALALNQTQHCKQLEGLVSAQVQLCRSNLELMHTVVHAAREVMKACRRAFADMRWNCSSIELAPNYLLDLERGTRESAFVYALSAAAISHAIARACTSGDLPGCSCGPVPGEPPGPGNRWGGCADNLSYGLLMGAKFSDAPMKVKKTGSQANKLMRLHNSEVGRQALRASLEMKCKCHGVSGSCSIRTCWKGLQELQDVAADLKTRYLSATKVVHRPMGTRKHLVPKDLDIRPVKDSELVYLQSSPDFCMKNEKVGSHGTQDRQCNKTSNGSDSCDLMCCGRGYNPYTDRVVERCHCKYHWCCYVTCRRCERTVERYVCKGRVLLRSSRESA

SEQ ID NO: 115 - protein, 12 aa, synthetic construct
GKIVNRGCRETA

SEQ ID NO: 116 - protein, 12 aa, synthetic construct
GRVLLRSSRESA

SEQ ID NO: 117 - protein, 12 aa, synthetic construct
GRAMLRSSREAA

SEQ ID NO: 118 - protein, 12 aa, synthetic construct
GPVLDKATRESA

SEQ ID NO: 119 - protein, 12 aa, synthetic construct
GPVLDKATRESA

SEQ ID NO: 120 - protein, 12 aa, synthetic construct
GKVVTQGTREAA

SEQ ID NO: 121 - protein, 12 aa, synthetic construct
GRVMQIGSRETA

SEQ ID NO: 122 - protein, 12 aa, synthetic construct
GRVMQIGSRETA

SEQ ID NO: 123 - protein, 12 aa, synthetic construct
GRVLQQDIRETA

SEQ ID NO: 124 - protein, 12 aa, synthetic construct
GKELKVGSREAA

SEQ ID NO: 125 - protein, 12 aa, synthetic construct
GQELRVGSREAA

SEQ ID NO: 126 - protein, 12 aa, synthetic construct
HNRLRAATRETS

SEQ ID NO: 127 - protein, 12 aa, synthetic construct
HGGLRSANRETA

SEQ ID NO: 128 - protein, 12 aa, synthetic construct
ASLLKRGFKETA

SEQ ID NO: 129 - protein, 12 aa, synthetic construct
TGLLQRGFKETA

SEQ ID NO: 130 - protein, 12 aa, synthetic construct
SPIFSRGFRESA

SEQ ID NO: 131 - protein, 12 aa, synthetic construct
SAILKRGFRESA

SEQ ID NO: 132 - protein, 12 aa, synthetic construct
GYELSSGTKETA

SEQ ID NO: 133 - protein, 18 aa, synthetic construct
DSLAIFGPVLDKATRESA

SEQ ID NO: 134 - protein, 10 aa, synthetic construct
DSLAIFRESA

SEQ ID NO: 135 - protein, 18 aa, synthetic construct
DSLAIFLLDLERGTRESA

SEQ ID NO: 136 - protein, 471 aa, synthetic construct
MGWSCIILFLVATATGVHSEVELVESGGGLVQPGRSLKLSCAASGFTFSDYGMAWVRQTPTKGLEWVASITSGGGNPYYRDSVKGRFTISRDNAKNTQHLQMDSLRSEDTATYYCARHEYYGNYMTCFDYWGQGVMVTVSSASTKGPSVFPLAPSSKSTSGGTAALGCLVKDYFPEPVTVSWNSGALTSGVHTFPAVLQSSGLYSLSSVVTVPSSSLGTQTYICNVNHKPSNTKVDKKVEPKSCDKTHTCPPCPAPELLGGPSVFLFPPKPKDTLMISRTPEVTCVVVDVSHEDPEVKFNWYVDGVEVHNAKTKPREEQYNSTYRVVSVLTVLHQDWLNGKEYKCKVSNKALPAPIEKTISKAKGQPREPQVYTLPPSRDELTKNQVSLTCLVKGFYPSDIAVEWESNGQPENNYKTTPPVLDSDGSFFLYSKLTVDKSRWQQGNVFSCSVMHEALHNHYTQKSLSLSPGK

SEQ ID NO: 137 - protein, 234 aa, synthetic construct
MGWSCIILFLVATATGVHSAIVLNQSPSSIVASQGEKVTITCRASLSISSNYLHWYQQKPGAFPKLVIYSTSYRASGVPSRFSGSGSGTSYSFTISRVEAEDVATYYCQQGSSDPLTFGSGTKLEIKRTVAAPSVFIFPPSDEQLKSGTASVVCLLNNFYPREAKVQWKVDNALQSGNSQESVTEQDSKDSTYSLSSTLTLSKADYEKHKVYACEVTHQGLSSPVTKSFNRGEC

SEQ ID NO: 138 - protein, 471 aa, synthetic construct
MGWSCIILFLVATATGVHSQVQLVESGGGVVQPGRSLRLSCAASGFTFSDYGMAWVRQAPGKGLEWVASITSGGGNPYYRDSVKGRFTISRDNSKNTLYLQMNSLRAEDTAVYYCARHEYYGNYMTCFDYWGQGTLVTVSSASTKGPSVFPLAPSSKSTSGGTAALGCLVKDYFPEPVTVSWNSGALTSGVHTFPAVLQSSGLYSLSSVVTVPSSSLGTQTYICNVNHKPSNTKVDKKVEPKSCDKTHTCPPCPAPELLGGPSVFLFPPKPKDTLMISRTPEVTCVVVDVSHEDPEVKFNWYVDGVEVHNAKTKPREEQYNSTYRVVSVLTVLHQDWLNGKEYKCKVSNKALPAPIEKTISKAKGQPREPQVYTLPPSRDELTKNQVSLTCLVKGFYPSDIAVEWESNGQPENNYKTTPPVLDSDGSFFLYSKLTVDKSRWQQGNVFSCSVMHEALHNHYTQKSLSLSPGK

SEQ ID NO: 139 - protein, 234 aa, synthetic construct
MGWSCIILFLVATATGVHSDIQMTQSPSSLSASVGDRVTITCRASLSISSNYLHWYQQKPGKAPKLLIYSTSYRASGVPSRFSGSGSGTDFTLTISSLQPEDFATYYCQQGSSDPLTFGGGTKLEIKRTVAAPSVFIFPPSDEQLKSGTASVVCLLNNFYPREAKVQWKVDNALQSGNSQESVTEQDSKDSTYSLSSTLTLSKADYEKHKVYACEVTHQGLSSPVTKSFNRGEC

SEQ ID NO: 140 - protein, 14 aa, synthetic construct
NYLLDLERGTRESA

SEQ ID NO: 141 - protein, 6 aa, synthetic construct
NYRESA

SEQ ID NO: 142 - protein, 19 aa, synthetic construct
DSLAIFGPVLDKATRESAC

SEQ ID NO: 143 - protein, 13 aa, synthetic construct
GKELKVGSREAAC

SEQ ID NO: 144 - protein, 13 aa, synthetic construct
GQELRVGSREAAC

SEQ ID NO: 145 - protein, 14 aa, synthetic construct
RASLLKRGFKETAC

SEQ ID NO: 146 - protein, 15 aa, synthetic construct
YESPIFSRGFRESAC